European Patent Application EP 4 371 997 A1, published May 22, 2024. Title: MUTANT OF PORIN MONOMER, PROTEIN PORE, AND USE THEREOF. Applicant: QITAN TECHNOLOGY LTD., CHENGDU. The sequence listing filed with the application follows.

SEQUENCE LISTING (30 sequences)

SEQ ID NO: 1 - protein, 283 aa, Pseudomonas taeanensis
MNRLLAMAMLLAALQGCALREPMPAELENATPTLTPRASTYYDLLALPRPKGRLVAAVYGFRDQTGQYKPTPASSFSTSVTQGAASMLVDALQASGWFRVLEREGLQNILTERKIIRASQNKPNTPVNIQADLPSLQAANILLEGGVIAYDTNVRSGGEGAAYLGISLSQEYRVDQVSVNLRAVDVRSGQVLANVMTSKTIYSVGRNAGIFKFIEFKELLEAEAGYTTNEPAQLCVLSAIEAAVAHLVAQGIERRLWQAADESSFDKSSLPKYMSQARADPLP

SEQ ID NO: 2 - DNA, 852 bp, Pseudomonas taeanensis
atgaacagactactagcgatggcgatgttgctggccgccctgcaaggctgcgccttgcgcgaacccatgccggcggagctggaaaacgcgactccgaccctgacgccgcgggcctcgacctattacgacttgctggccctgccgcggcccaaaggccgcctggttgccgctgtgtacggcttccgcgaccagactgggcagtacaagccgacgcctgccagttcgttctccaccagcgtgactcagggcgccgccagcatgctggtcgacgcgttgcaggccagcggctggttccgggtgctggagcgcgagggcctgcagaatatcctgaccgaacgcaagatcattcgcgcctcgcagaacaagcccaataccccggtgaatatccaggccgatctgccctcgttgcaggccgccaacatccttctggaaggcggggtgatcgcctacgacactaatgtacgtagcggtggtgagggggctgcctacctgggtatcagcctgtctcaggagtatcgggtggatcaggtttcggtgaacctgcgtgcggtggatgtgcgcagcggtcaggtactggccaacgtcatgacctccaagaccatctattcggtcgggcgcaatgccggcatattcaaattcatcgagttcaaggagctgttggaggccgaggcgggctacacgaccaatgaaccggcgcagctgtgtgtgctctcggctatcgaagccgccgtggctcatctggtggcccagggcatcgagcggcgcctgtggcaggctgctgacgaaagctccttcgataagtcgtcactgcccaagtacatgagccaggcgcgggccgatccactgccttag

SEQ ID NO: 3 - DNA, 10 bp, Artificial Sequence
  part of BS7-4C3-SE1
tttttttttt

SEQ ID NO: 4 - DNA, 28 bp, Artificial Sequence
  part of BS7-4C3-SE1
aatgtacttcgttcagttacgtattgct

SEQ ID NO: 5 - DNA, 42 bp, Artificial Sequence
  part of BS7-4C3-SE1
gcaatacgtaactgaacgaagttcactatcgcattctcatga

SEQ ID NO: 6 - DNA, 20 bp, Artificial Sequence
  part of BS7-4C3-SE1
tcatgagaatgcgatagtga

SEQ ID NO: 7 - DNA, 89 bp, Artificial Sequence
  part of BS7-4C3-SE1
aaaaaaaaaaaaaaaaaaaaaaaaaaaaaaaaaaaaaaaaaagcaatacgtaactgaacgaagtacattaaaaaaaaaaaaaaaaaaaa

SEQ ID NO: 8 - DNA, 24 bp, Artificial Sequence
  part of BS7-4C3-SE1
atcctttttttttttttttttttt

SEQ ID NO: 9 - DNA, 48 bp, Artificial Sequence
  part of BS7-4C3-SE1
aatgtacttcgttcagttacgtattgcttttttttttttttttttttt

SEQ ID NO: 10 - DNA, 20 bp, Artificial Sequence
  part of BS7-4C3-SE1
tttttttttttttttttttt

SEQ ID NO: 11 - DNA, 10 bp, Artificial Sequence
  part of BS7-4C3-PLT
tttttttttt

SEQ ID NO: 12 - DNA, 28 bp, Artificial Sequence
  part of BS7-4C3-PLT
aatgtacttcgttcagttacgtattgct

SEQ ID NO: 13 - DNA, 42 bp, Artificial Sequence; identical to SEQ ID NO: 5
  part of BS7-4C3-PLT

SEQ ID NO: 14 - DNA, 20 bp, Artificial Sequence
  part of BS7-4C3-PLT
tcatgagaatgcgatagtga

SEQ ID NO: 15 - DNA, 28 bp, Artificial Sequence
  part of BS7-4C3-PLT
aaaaaaaaaaaaaaaaaaaaaaaaaaaa

SEQ ID NO: 16 - DNA, 12 bp, Artificial Sequence
  part of BS7-4C3-PLT
aaaaaaaaaaaa

SEQ ID NO: 17 - DNA, 132 bp, Artificial Sequence
  part of BS7-4C3-PLT
aaaaaaaaaaaaaatctctgaatctctgaatctctgaatctctaaaaaaaaaaaagaaaaaaaaaaaacaaaaaaaaaaaataaaaaaaaaaaaagcaatacgtaactgaacgaagtacattaaaaaaaaaa

SEQ ID NO: 18 - DNA, 42 bp, Artificial Sequence
  part of BS7-4C3-PLT
atccttttttttttaatgtacttcgttcagttacgtattgct

SEQ ID NO: 19 - DNA, 94 bp, Artificial Sequence
  part of BS7-4C3-PLT
ttttttttttttattttttttttttgttttttttttttcttttttttttttagagattcagagattcagagattcagagatttttttttttttt

SEQ ID NO: 20 - DNA, 12 bp, Artificial Sequence
  part of BS7-4C3-PLT
tttttttttttt

SEQ ID NO: 21 - DNA, 28 bp, Artificial Sequence
  part of BS7-4C3-PLT
tttttttttttttttttttttttttttt

SEQ ID NO: 22 - protein, 441 aa, Artificial Sequence
  helicase
MITIDQLTEGQFDSLQRAKVLIQEATKNDGNWNHRTKHLTINGPAGTGKTTMMKFLVSWLRDEGITGVALAAPTHAAKKVLANAVGEEVSTIHSILKINPTTYECKQFFEQSAPPDLSKIRILICEECSFYDIKLFEILMNSIQPWTIIIGIGDRAQLRPADDKGISRFFTDQRFEQTYLTEIKRSNMPIIEVATEIRNGGWIRENIIDDLGVKQDKSVSEFMTNYFKVVKSIDDLYETRMYAYTNNSVDTLNKIIRKKLYETEQDFIVGEPIVMQEPLIRDINYEGKRFQEIVFNNGEYLEVSEIKPMESVLKCRNIDYQLVLHYYQLKVKSIDTGESGLINTISDKNELNKFYMFLGKVCQDYKSGTIKAFWDDFWKIKNNYHRVKPLPVSTIHKGQGSTVDNSFLYTPCITKYAEPDLASQLLYVGVTRARHNVNFVG

SEQ ID NO: 23 - DNA, 1326 bp, Artificial Sequence
  helicase
atgatcaccatcgaccagctgaccgaaggtcagttcgactctctgcagcgtgctaaagttctgatccaggaagctaccaaaaacgacggtaactggaaccaccgtaccaaacacctgaccatcaacggtccggctggtaccggtaaaaccaccatgatgaaattcctggtttcttggctgcgtgacgaaggtatcaccggtgttgctctggctgctccgacccacgctgctaaaaaagttctggctaacgctgttggtgaagaagtttctaccatccactctatcctgaaaatcaacccgaccacctacgaatgcaaacagttcttcgaacagtctgctccgccggacctgtctaaaatccgtatcctgatctgcgaagaatgctctttctacgacatcaaactgttcgaaatcctgatgaactctatccagccgtggaccatcatcatcggtatcggtgaccgtgctcagctgcgtccggctgacgacaaaggtatctctcgtttcttcaccgaccagcgtttcgaacagacctacctgaccgaaatcaaacgttctaacatgccgatcatcgaagttgctaccgaaatccgtaacggtggttggattcgtgaaaacatcatcgacgacctgggtgttaaacaggacaaatctgtttctgaatttatgaccaactacttcaaagttgttaaatctatcgacgacctgtacgaaacccgtatgtacgcttacaccaacaactctgttgacaccctgaacaaaatcatccgtaaaaaactgtacgaaaccgaacaggacttcatcgttggtgaaccgatcgttatgcaggaaccgctgatccgtgacatcaactacgaaggtaaacgtttccaggaaatcgttttcaacaacggtgaatacctggaagtttctgaaatcaaaccgatggaatctgttctgaaatgccgtaacatcgactaccagctggttctgcactactaccagctgaaagttaaatctatcgacaccggtgaatctggtctgatcaacaccatctctgacaaaaacgaactgaacaaattctacatgttcctgggtaaagtttgccaggactacaaatctggtaccatcaaagcgttctgggacgacttctggaaaatcaaaaacaactaccaccgtgttaaaccgctgccggtttctaccatccacaaaggtcagggttctaccgttgacaactctttcctgtacaccccgtgcatcaccaaatacgctgaaccggacctggcttctcagctgctgtacgttggtgttacccgtgctcgtcacaacgttaacttcgttggttaa

SEQ ID NO: 24 - protein, 283 aa, Artificial Sequence
  mutant 1
MNRLLAMAMLLAALQGCALREPMPAELENATPTLTPRASTYYDLLALPRPKGRLVAAVYGFRDQTGQYRPSPASAQSTSVTQGAASMLVDALQASGWFRVLEREGLQNILTERKIIRASQNKPNTPVNIQADLPSLQAANILLEGGVIAYDTNVRSGGEGAAYLGISLSQEYRVDQVSVNLRAVDVRSGQVLANVMTSKTIYSVGRNAGIFKFIEFKELLEAEAGYTTNEPAQLCVLSAIEAAVAHLVAQGIERRLWQAADESSFDKSSLPKYMSQARADPLP

SEQ ID NO: 25 - DNA, 849 bp, Artificial Sequence
  mutant 1
atgaataggttgttagcaatggctatgctattggcggctttgcaaggttgtgcactgcgtgaaccgatgccggcagaattggagaacgcgaccccgaccctgacgccacgtgcgtctacgtactacgacctgctggctctcccgcgtccgaagggtcgcctggtggcggcggtgtatggttttcgcgatcagactggtcagtaccgtccgtccccggcgtcagcacaaagcaccagcgtcacccagggtgcagcgtctatgctggttgacgcattacaagcgtccggctggttccgcgtgctggagcgcgaaggcctgcaaaacatccttacggaacgtaaaatcattcgtgcatctcagaacaaaccgaataccccagttaatatccaagcggatctgccttcgttgcaggcggcgaacattctgctcgagggtggcgtgattgcatacgacaccaatgttcgttctggcggtgaaggcgctgcgtacctgggtatcagcctgtcccaagaatatcgcgttgaccaggttagcgttaacctgcgtgcggttgatgtccgtagcggccaagtactggcgaacgtgatgacctcgaaaaccatttatagcgtgggtcgtaatgccggcatttttaagttcatcgaattcaaagagttgttggaggcagaagcgggttataccacaaacgagccggcccaactttgcgttctgagcgcaatcgaggcggctgtggcccacctggtcgcgcagggcatcgagcgccgtctgtggcaggctgccgatgagagctcctttgataagagcagcttgccgaagtacatgagccaggcgagagccgacccgctgccg

SEQ ID NO: 26 - protein, 283 aa, Artificial Sequence
  mutant 2
MNRLLAMAMLLAALQGCALREPMPAELENATPTLTPRASTYYDLLALPRPKGRLVAAVYGFRDQTGQYKPGPASTKSTSVTQGAASMLVDALQASGWFRVLEREGLQNILTERKIIRASQNKPNTPVNIQADLPSLQAANILLEGGVIAYDTNVRSGGEGAAYLGISLSQEYRVDQVSVNLRAVDVRSGQVLANVMTSKTIYSVGRNAGIFKFIEFKELLEAEAGYTTNEPAQLCVLSAIEAAVAHLVAQGIERRLWQAADESSFDKSSLPKYMSQARADPLP

SEQ ID NO: 27 - protein, 283 aa, Artificial Sequence
  mutant 3
MNRLLAMAMLLAALQGCALREPMPAELENATPTLTPRASTYYDLLALPRPKGRLVAAVYGFRDLTGQYRPSPASANSTAVTQGAASMLVDALQASGWFRVLEREGLQNILTERKIIRASQNKPNTPVNIQADLPSLQAANILLEGGVIAYDTNVRSGGEGAAYLGISLSQEYRVDQVSVNLRAVDVRSGQVLANVMTSKTIYSVGRNAGIFKFIEFKELLEAEAGYTTNEPAQLCVLSAIEAAVAHLVAQGIERRLWQAADESSFDKSSLPKYMSQARADPLP

SEQ ID NO: 28 - protein, 283 aa, Artificial Sequence
  mutant 4
MNRLLAMAMLLAALQGCALREPMPAELENATPTLTPRASTYYDLLALPRPKGRLVAAVYGFRDLTGQYRPSPASALSTAVTQGAASMLVDALQASGWFRVLEREGLQNILTERKIIRASQNKPNTPVNIQADLPSLQAANILLEGGVIAYDTNVRSGGEGAAYLGISLSQEYRVDQVSVNLRAVDVRSGQVLANVMTSKTIYSVGRNAGIFKFIEFKELLEAEAGYTTNEPAQLCVLSAIEAAVAHLVAQGIERRLWQAADESSFDKSSLPKYMSQARADPLP

SEQ ID NO: 29 - protein, 283 aa, Artificial Sequence
  mutant 5
MNRLLAMAMLLAALQGCALREPMPAELENATPTLTPRASTYYDLLALPRPKGRLVAAVYGFSVQTGQFRPSPASAQSTSVTQGAASMLVDALQASGWFRVLERVGLQNILTERKIIRASQNKPNTPVNIQADLPSLQAANILLEGGVIAYDTNVRSGGEGAAYLGISLSQEYRVDQVSVNLRAVDVRSGQVLANVMTSKTIYSVGRNAGIFKFIEFKELLEAEAGYTTNEPAQLCVLSAIEAAVAHLVAQGIERRLWQAADESSFDKSSLPKYMSQARADPLP

SEQ ID NO: 30 - protein, 283 aa, Artificial Sequence
  mutant 6
MNRLLAMAMLLAALQGCALREPMPAELENATPTLTPRASTYYDLLALPRPKGRLVAAVYGFRDQTGQFRPSPASAQSTSVTQGAASMLVDALQASGWFRVLEREGLQNILTERKIIRASQNKPNTPVNIQADLPSLQAANILLEGGVIAYDTNVRSGGEGAAYLGISLSQNYRVNQVSVNLRAVDVRSGQVLANVMTSKTIYSVGRNAGIFKFIEFKELLEAEAGYTTNEPAQLCVLSAIEAAVAHLVAQGIERRLWQAADESSFDKSSLPKYMSQARADPLP